European Patent Application EP 4 289 484 A2, published December 13, 2023. Title: ANTI-CTLA-4 ANTIBODIES AND METHODS OF USE THEREOF. Applicant: AGENUS INC. Application EP. The sequence listing filed with the application follows.

SEQUENCE LISTING (52 sequences)

SEQ ID NO: 1 - protein, 118 aa, synthetic construct
  REGION 1..118: note = source = /note="Description of Artificial Sequence: Synthetic polypeptide"
EVQLVESGGGLVKPGGSLRLSCAASGFTFSSYSMNWVRQAPGKGLEWVSSISSSSSYIYYADSVKGRFTISRDNAKNSLYLQMNSLRAEDTAVYYCARVGLMGPFDIWGQGTMVTVSS

SEQ ID NO: 2 - protein, 118 aa, synthetic construct
  REGION 1..118: note = source = /note="Description of Artificial Sequence: Synthetic polypeptide"
EVQLVESGGGLVKPGGSLRLSCAASGFTFSSYSMNWVRQAPGKGLEWVSSISSSSSYIYYADSVKGRFTISRDNAKNSLYLQMNSLRAEDTAVYYCARVGLFGPFDIWGQGTMVTVSS

SEQ ID NO: 3 - protein, 118 aa, synthetic construct
  REGION 1..118: note = source = /note="Description of Artificial Sequence: Synthetic polypeptide"
EVQLVESGGGLVKPGGSLRLSCAASGFTFSSYSMNWVRQAPGKGLEWVSSISSSSSYIYYADSVKGRFTISRDNAKNSLYLQMNSLRAEDTAVYYCARVGLMGPFDIWGQGTLVTVSS

SEQ ID NO: 4 - protein, 118 aa, synthetic construct
  REGION 1..118: note = source = /note="Description of Artificial Sequence: Synthetic polypeptide"
EVQLVESGGGLVKPGGSLRLSCAASGFTFSSYSMNWVRQAPGKGLEWVSSISSSSSYIYYAESVKGRFTISRDNAKNSLYLQMNSLRAEDTAVYYCARVGLMGPFDIWGQGTMVTVSS

SEQ ID NO: 5 - protein, 118 aa, synthetic construct
  REGION 1..118: note = source = /note="Description of Artificial Sequence: Synthetic polypeptide"
EVQLVESGGGLVKPGGSLRLSCAASGFTFSSYSMNWVRQAPGKGLEWVSSISSSSSYIYYADSVKGRFTISRDNAKNSLYLQMNSLRAEDTAVYYCARVGLFGPFDIWGQGTLVTVSS

SEQ ID NO: 6 - protein, 118 aa, synthetic construct
  REGION 1..118: note = source = /note="Description of Artificial Sequence: Synthetic polypeptide"
EVQLVESGGGLVKPGGSLRLSCAASGFTFSSYSMNWVRQAPGKGLEWVSSISSSSSYIYYAESVKGRFTISRDNAKNSLYLQMNSLRAEDTAVYYCARVGLFGPFDIWGQGTMVTVSS

SEQ ID NO: 7 - protein, 118 aa, synthetic construct
  REGION 1..118: note = source = /note="Description of Artificial Sequence: Synthetic polypeptide"
EVQLVESGGGLVKPGGSLRLSCAASGFTFSSYSMNWVRQAPGKGLEWVSSISSSSSYIYYAESVKGRFTISRDNAKNSLYLQMNSLRAEDTAVYYCARVGLMGPFDIWGQGTLVTVSS

SEQ ID NO: 8 - protein, 118 aa, synthetic construct
  REGION 1..118: note = source = /note="Description of Artificial Sequence: Synthetic polypeptide"
EVQLVESGGGLVKPGGSLRLSCAASGFTFSSYSMNWVRQAPGKGLEWVSSISSSSSYIYYAESVKGRFTISRDNAKNSLYLQMNSLRAEDTAVYYCARVGLFGPFDIWGQGTLVTVSS

SEQ ID NO: 9 - protein, 107 aa, synthetic construct
  REGION 1..107: note = source = /note="Description of Artificial Sequence: Synthetic polypeptide"
EIVLTQSPGTLSLSPGERATLSCRASQSVSRYLGWYQQKPGQAPRLLIYGASTRATGIPDRFSGSGSGTDFTLTITRLEPEDFAVYYCQQYGSSPWTFGQGTKVEIK

SEQ ID NO: 10 - protein, 5 aa, synthetic construct
  REGION 1..5: note = source = /note="Description of Artificial Sequence: Synthetic peptide"
SYSMN

SEQ ID NO: 11 - protein, 17 aa, synthetic construct
  REGION 1..17: note = source = /note="Description of Artificial Sequence: Synthetic peptide"
SISSSSSYIYYADSVKG

SEQ ID NO: 12 - protein, 17 aa, synthetic construct
  REGION 1..17: note = source = /note="Description of Artificial Sequence: Synthetic peptide"
SISSSSSYIYYAESVKG

SEQ ID NO: 13 - protein, 9 aa, synthetic construct
  REGION 1..9: note = source = /note="Description of Artificial Sequence: Synthetic peptide"
VGLMGPFDI

SEQ ID NO: 14 - protein, 9 aa, synthetic construct
  REGION 1..9: note = source = /note="Description of Artificial Sequence: Synthetic peptide"
VGLFGPFDI

SEQ ID NO: 15 - protein, 11 aa, synthetic construct
  REGION 1..11: note = source = /note="Description of Artificial Sequence: Synthetic peptide"
RASQSVSRYLG

SEQ ID NO: 16 - protein, 7 aa, synthetic construct
  REGION 1..7: note = source = /note="Description of Artificial Sequence: Synthetic peptide"
GASTRAT

SEQ ID NO: 17 - protein, 9 aa, synthetic construct
  REGION 1..9: note = source = /note="Description of Artificial Sequence: Synthetic peptide"
QQYGSSPWT

SEQ ID NO: 18 - protein, 17 aa, synthetic construct
  VARIANT 13: note = /replace="Asp"
  REGION 1..17: note = MISC_FEATURE - /note="Variant residues given in the sequence have no preference with respect to those in the annotations for variant positions"
  REGION 1..17: note = source = /note="Description of Artificial Sequence: Synthetic peptide"
SISSSSSYIYYAESVKG

SEQ ID NO: 19 - protein, 9 aa, synthetic construct
  VARIANT 4: note = /replace="Met"
  REGION 1..9: note = MISC_FEATURE - /note="Variant residues given in the sequence have no preference with respect to those in the annotations for variant positions"
  REGION 1..9: note = source = /note="Description of Artificial Sequence: Synthetic peptide"
VGLFGPFDI

SEQ ID NO: 20 - protein, 118 aa, synthetic construct; identical to SEQ ID NO: 8
  VARIANT 62: note = /replace="Asp"
  VARIANT 102: note = /replace="Met"
  VARIANT 113: note = /replace="Met"
  REGION 1..118: note = MISC_FEATURE - /note="Variant residues given in the sequence have no preference with respect to those in the annotations for variant positions"
  REGION 1..118: note = source = /note="Description of Artificial Sequence: Synthetic polypeptide"

SEQ ID NO: 21 - protein, 98 aa, Homo sapiens
EVQLVESGGGLVKPGGSLRLSCAASGFTFSSYSMNWVRQAPGKGLEWVSSISSSSSYIYYADSVKGRFTISRDNAKNSLYLQMNSLRAEDTAVYYCAR

SEQ ID NO: 22 - protein, 96 aa, Homo sapiens
EIVLTQSPGTLSLSPGERATLSCRASQSVSSSYLAWYQQKPGQAPRLLIYGASSRATGIPDRFSGSGSGTDFTLTISRLEPEDFAVYYCQQYGSSP

SEQ ID NO: 23 - protein, 447 aa, synthetic construct
  REGION 1..447: note = source = /note="Description of Artificial Sequence: Synthetic polypeptide"
EVQLVESGGGLVKPGGSLRLSCAASGFTFSSYSMNWVRQAPGKGLEWVSSISSSSSYIYYAESVKGRFTISRDNAKNSLYLQMNSLRAEDTAVYYCARVGLFGPFDIWGQGTLVTVSSASTKGPSVFPLAPSSKSTSGGTAALGCLVKDYFPEPVTVSWNSGALTSGVHTFPAVLQSSGLYSLSSVVTVPSSSLGTQTYICNVNHKPSNTKVDKRVEPKSCDKTHTCPPCPAPELLGGPSVFLFPPKPKDTLMISRTPEVTCVVVDVSHEDPEVKFNWYVDGVEVHNAKTKPREEQYNSTYRVVSVLTVLHQDWLNGKEYKCKVSNKALPAPIEKTISKAKGQPREPQVYTLPPSREEMTKNQVSLTCLVKGFYPSDIAVEWESNGQPENNYKTTPPVLDSDGSFFLYSKLTVDKSRWQQGNVFSCSVMHEALHNHYTQKSLSLSPG

SEQ ID NO: 24 - protein, 447 aa, synthetic construct
  REGION 1..447: note = source = /note="Description of Artificial Sequence: Synthetic polypeptide"
EVQLVESGGGLVKPGGSLRLSCAASGFTFSSYSMNWVRQAPGKGLEWVSSISSSSSYIYYAESVKGRFTISRDNAKNSLYLQMNSLRAEDTAVYYCARVGLFGPFDIWGQGTLVTVSSASTKGPSVFPLAPSSKSTSGGTAALGCLVKDYFPEPVTVSWNSGALTSGVHTFPAVLQSSGLYSLSSVVTVPSSSLGTQTYICNVNHKPSNTKVDKRVEPKSCDKTHTCPPCPAPELLGGPDVFLFPPKPKDTLMISRTPEVTCVVVDVSHEDPEVKFNWYVDGVEVHNAKTKPREEQYNSTYRVVSVLTVLHQDWLNGKEYKCKVSNKALPAPEEKTISKAKGQPREPQVYTLPPSREEMTKNQVSLTCLVKGFYPSDIAVEWESNGQPENNYKTTPPVLDSDGSFFLYSKLTVDKSRWQQGNVFSCSVMHEALHNHYTQKSLSLSPG

SEQ ID NO: 25 - protein, 447 aa, synthetic construct
  REGION 1..447: note = source = /note="Description of Artificial Sequence: Synthetic polypeptide"
EVQLVESGGGLVKPGGSLRLSCAASGFTFSSYSMNWVRQAPGKGLEWVSSISSSSSYIYYAESVKGRFTISRDNAKNSLYLQMNSLRAEDTAVYYCARVGLFGPFDIWGQGTLVTVSSASTKGPSVFPLAPSSKSTSGGTAALGCLVKDYFPEPVTVSWNSGALTSGVHTFPAVLQSSGLYSLSSVVTVPSSSLGTQTYICNVNHKPSNTKVDKRVEPKSCDKTHTCPPCPAPELLGGPDVFLFPPKPKDTLMISRTPEVTCVVVDVSHEDPEVKFNWYVDGVEVHNAKTKPREEQYNSTYRVVSVLTVLHQDWLNGKEYKCKVSNKALPLPEEKTISKAKGQPREPQVYTLPPSREEMTKNQVSLTCLVKGFYPSDIAVEWESNGQPENNYKTTPPVLDSDGSFFLYSKLTVDKSRWQQGNVFSCSVMHEALHNHYTQKSLSLSPG

SEQ ID NO: 26 - protein, 447 aa, synthetic construct
  REGION 1..447: note = source = /note="Description of Artificial Sequence: Synthetic polypeptide"
EVQLVESGGGLVKPGGSLRLSCAASGFTFSSYSMNWVRQAPGKGLEWVSSISSSSSYIYYAESVKGRFTISRDNAKNSLYLQMNSLRAEDTAVYYCARVGLFGPFDIWGQGTLVTVSSASTKGPSVFPLAPSSKSTSGGTAALGCLVKDYFPEPVTVSWNSGALTSGVHTFPAVLQSSGLYSLSSVVTVPSSSLGTQTYICNVNHKPSNTKVDKRVEPKSCDKTHTCPPCPAPELVGGPSVFLLPPKPKDTLMISRTPEVTCVVVDVSHEDPEVKFNWYVDGVEVHNAKTKPPEEQYNSTLRVVSVLTVLHQDWLNGKEYKCKVSNKALPAPIEKTISKAKGQPREPQVYTLPPSREEMTKNQVSLTCLVKGFYPSDIAVEWESNGQPENNYKTTPLVLDSDGSFFLYSKLTVDKSRWQQGNVFSCSVMHEALHNHYTQKSLSLSPG

SEQ ID NO: 27 - protein, 214 aa, synthetic construct
  REGION 1..214: note = source = /note="Description of Artificial Sequence: Synthetic polypeptide"
EIVLTQSPGTLSLSPGERATLSCRASQSVSRYLGWYQQKPGQAPRLLIYGASTRATGIPDRFSGSGSGTDFTLTITRLEPEDFAVYYCQQYGSSPWTFGQGTKVEIKRTVAAPSVFIFPPSDEQLKSGTASVVCLLNNFYPREAKVQWKVDNALQSGNSQESVTEQDSKDSTYSLSSTLTLSKADYEKHKVYACEVTHQGLSSPVTKSFNRGEC

SEQ ID NO: 28 - protein, 329 aa, Homo sapiens
ASTKGPSVFPLAPSSKSTSGGTAALGCLVKDYFPEPVTVSWNSGALTSGVHTFPAVLQSSGLYSLSSVVTVPSSSLGTQTYICNVNHKPSNTKVDKRVEPKSCDKTHTCPPCPAPELLGGPSVFLFPPKPKDTLMISRTPEVTCVVVDVSHEDPEVKFNWYVDGVEVHNAKTKPREEQYNSTYRVVSVLTVLHQDWLNGKEYKCKVSNKALPAPIEKTISKAKGQPREPQVYTLPPSREEMTKNQVSLTCLVKGFYPSDIAVEWESNGQPENNYKTTPPVLDSDGSFFLYSKLTVDKSRWQQGNVFSCSVMHEALHNHYTQKSLSLSPG

SEQ ID NO: 29 - protein, 329 aa, synthetic construct
  REGION 1..329: note = source = /note="Description of Artificial Sequence: Synthetic polypeptide"
ASTKGPSVFPLAPSSKSTSGGTAALGCLVKDYFPEPVTVSWNSGALTSGVHTFPAVLQSSGLYSLSSVVTVPSSSLGTQTYICNVNHKPSNTKVDKRVEPKSCDKTHTCPPCPAPELLGGPDVFLFPPKPKDTLMISRTPEVTCVVVDVSHEDPEVKFNWYVDGVEVHNAKTKPREEQYNSTYRVVSVLTVLHQDWLNGKEYKCKVSNKALPAPEEKTISKAKGQPREPQVYTLPPSREEMTKNQVSLTCLVKGFYPSDIAVEWESNGQPENNYKTTPPVLDSDGSFFLYSKLTVDKSRWQQGNVFSCSVMHEALHNHYTQKSLSLSPG

SEQ ID NO: 30 - protein, 329 aa, synthetic construct
  REGION 1..329: note = source = /note="Description of Artificial Sequence: Synthetic polypeptide"
ASTKGPSVFPLAPSSKSTSGGTAALGCLVKDYFPEPVTVSWNSGALTSGVHTFPAVLQSSGLYSLSSVVTVPSSSLGTQTYICNVNHKPSNTKVDKRVEPKSCDKTHTCPPCPAPELLGGPDVFLFPPKPKDTLMISRTPEVTCVVVDVSHEDPEVKFNWYVDGVEVHNAKTKPREEQYNSTYRVVSVLTVLHQDWLNGKEYKCKVSNKALPLPEEKTISKAKGQPREPQVYTLPPSREEMTKNQVSLTCLVKGFYPSDIAVEWESNGQPENNYKTTPPVLDSDGSFFLYSKLTVDKSRWQQGNVFSCSVMHEALHNHYTQKSLSLSPG

SEQ ID NO: 31 - protein, 329 aa, synthetic construct
  REGION 1..329: note = source = /note="Description of Artificial Sequence: Synthetic polypeptide"
ASTKGPSVFPLAPSSKSTSGGTAALGCLVKDYFPEPVTVSWNSGALTSGVHTFPAVLQSSGLYSLSSVVTVPSSSLGTQTYICNVNHKPSNTKVDKRVEPKSCDKTHTCPPCPAPELVGGPSVFLLPPKPKDTLMISRTPEVTCVVVDVSHEDPEVKFNWYVDGVEVHNAKTKPPEEQYNSTLRVVSVLTVLHQDWLNGKEYKCKVSNKALPAPIEKTISKAKGQPREPQVYTLPPSREEMTKNQVSLTCLVKGFYPSDIAVEWESNGQPENNYKTTPLVLDSDGSFFLYSKLTVDKSRWQQGNVFSCSVMHEALHNHYTQKSLSLSPG

SEQ ID NO: 32 - protein, 107 aa, synthetic construct [sequence omitted]

SEQ ID NO: 33 - protein, 223 aa, Homo sapiens
MACLGFQRHKAQLNLATRTWPCTLLFFLLFIPVFCKAMHVAQPAVVLASSRGIASFVCEYASPGKATEVRVTVLRQADSQVTEVCAATYMMGNELTFLDDSICTGTSSGNQVNLTIQGLRAMDTGLYICKVELMYPPPYYLGIGNGTQIYVIDPEPCPDSDFLLWILAAVSSGLFFYSFLLTAVSLSKMLKKRSPLTTGVYVKMPPTEPECEKQFQPYFIPIN

SEQ ID NO: 34 - protein, 4 aa, Homo sapiens
YLGI

SEQ ID NO: 35 - protein, 9 aa, Homo sapiens
YPPPYYLGI

SEQ ID NO: 36 - protein, 10 aa, Homo sapiens
YLGIGNGTQI

SEQ ID NO: 37 - protein, 15 aa, Homo sapiens
YPPPYYLGIGNGTQI

SEQ ID NO: 38 - protein, 7 aa, Homo sapiens
MYPPPYY

SEQ ID NO: 39 - skipped

SEQ ID NO: 40 - protein, 223 aa, Macaca fascicularis
MACLGFQRHKARLNLATRTRPYTLLFSLLFIPVFSKAMHVAQPAVVLANSRGIASFVCEYASPGKATEVRVTVLRQADSQVTEVCAATYMMGNELTFLDDSICTGTSSGNQVNLTIQGLRAMDTGLYICKVELMYPPPYYMGIGNGTQIYVIDPEPCPDSDFLLWILAAVSSGLFFYSFLLTAVSLSKMLKKRSPLTTGVYVKMPPTEPECEKQFQPYFIPIN

SEQ ID NO: 41 - protein, 223 aa, Mus musculus
MACLGLRRYKAQLQLPSRTWPFVALLTLLFIPVFSEAIQVTQPSVVLASSHGVASFPCEYSPSHNTDEVRVTVLRQTNDQMTEVCATTFTEKNTVGFLDYPFCSGTFNESRVNLTIQGLRAVDTGLYLCKVELMYPPPYFVGMGNGTQIYVIDPEPCPDSDFLLWILVAVSLGLFFYSFLVSAVSLSKMLKKRSPLTTGVYVKMPPTEPECEKQFQPYFIPIN

SEQ ID NO: 42 - protein, 223 aa, Rattus norvegicus
MACLGLQRYKTHLQLPSRTWPFGVLLSLLFIPIFSEAIQVTQPSVVLASSHGVASFPCEYASSHNTDEVRVTVLRQTNDQVTEVCATTFTVKNTLGFLDDPFCSGTFNESRVNLTIQGLRAADTGLYFCKVELMYPPPYFVGMGNGTQIYVIDPEPCPDSDFLLWILAAVSSGLFFYSFLVTAVSLNRTLKKRSPLTTGVYVKMPPTEPECEKQFQPYFIPIN

SEQ ID NO: 43 - protein, 220 aa, Homo sapiens
MLRLLLALNLFPSIQVTGNKILVKQSPMLVAYDNAVNLSCKYSYNLFSREFRASLHKGLDSAVEVCVVYGNYSQQLQVYSKTGFNCDGKLGNESVTFYLQNLYVNQTDIYFCKIEVMYPPPYLDNEKSNGTIIHVKGKHLCPSPLFPGPSKPFWVLVVVGGVLACYSLLVTVAFIIFWVRSKRSRLLHSDYMNMTPRRPGPTRKHYQPYAPPRDFAAYRS

SEQ ID NO: 44 - protein, 199 aa, Homo sapiens
MKSGLWYFFLFCLRIKVLTGEINGSANYEMFIFHNGGVQILCKYPDIVQQFKMQLLKGGQILCDLTKTKGSGNTVSIKSLKFCHSQLSNNSVSFFLYNLDHSHANYYFCNLSIFDPPPFKVTLTGGYLHIYESQLCCQLKFWLPIGCAAFVVVCILGCILICWLTKKKYSSSVHDPNGEYMFMRAVNTAKKSRLTDVTL

SEQ ID NO: 45 - protein, 289 aa, Homo sapiens
MKTLPAMLGTGKLFWVFFLIPYLDIWNIHGKESCDVQLYIKRQSEHSILAGDPFELECPVKYCANRPHVTWCKLNGTTCVKLEDRQTSWKEEKNISFFILHFEPVLPNDNGSYRCSANFQSNLIESHSTTLYVTDVKSASERPSKDEMASRPWLLYRLLPLGGLPLLITTCFCLFCCLRRHQGKQNELSDTAGREINLVDAHLKSEQTEASTRQNSQVLLSETGIYDNDPDLCFRMQEGSEVYSNPCLEENKPGIVYASLNHSVIGPNSRLARNVKEAPTEYASICVRS

SEQ ID NO: 46 - protein, 288 aa, Homo sapiens
MQIPQAPWPVVWAVLQLGWRPGWFLDSPDRPWNPPTFSPALLVVTEGDNATFTCSFSNTSESFVLNWYRMSPSNQTDKLAAFPEDRSQPGQDCRFRVTQLPNGRDFHMSVVRARRNDSGTYLCGAISLAPKAQIKESLRAELRVTERRAEVPTAHPSPSPRPAGQFQTLVVGVVGGLLGSLVLLVWVLAVICSRAARGTIGARRTGQPLKEDPSAVPVFSVDYGELDFQWREKTPEPPVPCVPEQTEYATIVFPSGMGTSSPARRGSADGPRSAQPLRPEDGHCSWPL

SEQ ID NO: 47 - protein, 447 aa, synthetic construct
  REGION 1..447: note = source = /note="Description of Artificial Sequence: Synthetic polypeptide"
EVQLVESGGGLVKPGGSLRLSCAASGFTFSSYSMNWVRQAPGKGLEWVSSISSSSSYIYYAESVKGRFTISRDNAKNSLYLQMNSLRAEDTAVYYCARVGLFGPFDIWGQGTLVTVSSASTKGPSVFPLAPSSKSTSGGTAALGCLVKDYFPEPVTVSWNSGALTSGVHTFPAVLQSSGLYSLSSVVTVPSSSLGTQTYICNVNHKPSNTKVDKRVEPKSCDKTHTCPPCPAPELLGGPSVFLFPPKPKDTLMISRTPEVTCVVVDVSHEDPEVKFNWYVDGVEVHNAKTKPREEQYASTYRVVSVLTVLHQDWLNGKEYKCKVSNKALPAPIEKTISKAKGQPREPQVYTLPPSREEMTKNQVSLTCLVKGFYPSDIAVEWESNGQPENNYKTTPPVLDSDGSFFLYSKLTVDKSRWQQGNVFSCSVMHEALHNHYTQKSLSLSPG

SEQ ID NO: 48 - protein, 447 aa, synthetic construct
  REGION 1..447: note = source = /note="Description of Artificial Sequence: Synthetic polypeptide"
EVQLVESGGGLVKPGGSLRLSCAASGFTFSSYSMNWVRQAPGKGLEWVSSISSSSSYIYYAESVKGRFTISRDNAKNSLYLQMNSLRAEDTAVYYCARVGLFGPFDIWGQGTLVTVSSASTKGPSVFPLAPSSKSTSGGTAALGCLVKDYFPEPVTVSWNSGALTSGVHTFPAVLQSSGLYSLSSVVTVPSSSLGTQTYICNVNHKPSNTKVDKRVEPKSCDKTHTCPPCPAPELLGGPSVFLFPPKPKDTLMISRTPEVTCVVVDVEHEDPEVKFNWYVDGVEVHNAKTKPREEQYNSTYRVVSVLTVLHQDWLNGKEYKCKVSNKAFPAPIEKTISKAKGQPREPQVYTLPPSREEMTKNQVSLTCLVKGFYPSDIAVEWESNGQPENNYKTTPPVLDSDGSFFLYSKLTVDKSRWQQGNVFSCSVMHEALHNHYTQKSLSLSPG

SEQ ID NO: 49 - protein, 446 aa, synthetic construct
  REGION 1..446: note = source = /note="Description of Artificial Sequence: Synthetic polypeptide"
EAKLQESGPVLVKPGASVKMSCKASGYTFTDYYMNWVKQSHGKSLEWIGVINPYNGDTSYNQKFKGKATLTVDKSSSTAYMELNSLTSEDSAVYYCARYYGSWFAYWGQGTLVTVSSAKTTAPSVYPLAPVCGDTTGSSVTLGCLVKGYFPEPVTLTWNSGSLSSGVHTFPAVLQSDLYTLSSSVTVTSSTWPSQSITCNVAHPASSTKVDKKIEPRGPTIKPCPPCKCPAPNLLGGPSVFIFPPKIKDVLMISLSPIVTCVVVDVSEDDPDVQISWFVNNVEVHTAQTQTHREDYNSTLRVVSALPIQHQDWMSGKEFKCKVNNKDLPAPIERTISKPKGSVRAPQVYVLPPPEEEMTKKQVTLTCMVTDFMPEDIYVEWTNNGKTELNYKNTEPVLDSDGSYFMYSKLRVEKKNWVERNSYSCSVVHEGLHNHHTTKSFSRTPG

SEQ ID NO: 50 - protein, 446 aa, synthetic construct
  REGION 1..446: note = source = /note="Description of Artificial Sequence: Synthetic polypeptide"
EAKLQESGPVLVKPGASVKMSCKASGYTFTDYYMNWVKQSHGKSLEWIGVINPYNGDTSYNQKFKGKATLTVDKSSSTAYMELNSLTSEDSAVYYCARYYGSWFAYWGQGTLVTVSSAKTTAPSVYPLAPVCGDTTGSSVTLGCLVKGYFPEPVTLTWNSGSLSSGVHTFPAVLQSDLYTLSSSVTVTSSTWPSQSITCNVAHPASSTKVDKKIEPRGPTIKPCPPCKCPAPNLLGGPDVFIFPPKIKDVLMISLSPIVTCVVVDVSEDDPDVQISWFVNNVEVHTAQTQTHREDYNSTLRVVSALPIQHQDWMSGKEFKCKVNNKDLPLPEERTISKPKGSVRAPQVYVLPPPEEEMTKKQVTLTCMVTDFMPEDIYVEWTNNGKTELNYKNTEPVLDSDGSYFMYSKLRVEKKNWVERNSYSCSVVHEGLHNHHTTKSFSRTPG

SEQ ID NO: 51 - protein, 446 aa, synthetic construct
  REGION 1..446: note = source = /note="Description of Artificial Sequence: Synthetic polypeptide"
EAKLQESGPVLVKPGASVKMSCKASGYTFTDYYMNWVKQSHGKSLEWIGVINPYNGDTSYNQKFKGKATLTVDKSSSTAYMELNSLTSEDSAVYYCARYYGSWFAYWGQGTLVTVSSAKTTAPSVYPLAPVCGDTTGSSVTLGCLVKGYFPEPVTLTWNSGSLSSGVHTFPAVLQSDLYTLSSSVTVTSSTWPSQSITCNVAHPASSTKVDKKIEPRGPTIKPCPPCKCPAPNLLGGPSVFIFPPKIKDVLMISLSPIVTCVVVDVSEDDPDVQISWFVNNVEVHTAQTQTHREDYASTLRVVSALPIQHQDWMSGKEFKCKVNNKDLPAPIERTISKPKGSVRAPQVYVLPPPEEEMTKKQVTLTCMVTDFMPEDIYVEWTNNGKTELNYKNTEPVLDSDGSYFMYSKLRVEKKNWVERNSYSCSVVHEGLHNHHTTKSFSRTPG

SEQ ID NO: 52 - protein, 219 aa, synthetic construct
  REGION 1..219: note = source = /note="Description of Artificial Sequence: Synthetic polypeptide"
DIVMTQTTLSLPVSLGDQASISCRSSQSIVHSNGNTYLEWYLQKPGQSPKLLIYKVSNRFSGVPDRFSGSGSGTDFTLKISRVEAEDLGVYYCFQGSHVPYTFGGGTKLEIKRADAAPTVSIFPPSSEQLTSGGASVVCFLNNFYPKDINVKWKIDGSERQNGVLNSWTDQDSKDSTYSMSSTLTLTKDEYERHNSYTCEATHKTSTSPIVKSFNRNEC